European Patent Specification EP 3 566 053 B1, published July 17, 2024. Title: BIOMARKERS FOR LUNG CANCER STEM CELLS. Applicant: Pan-Chyr Yang Huei-Wen Chen Wan-Jiun Chen. The sequence listing filed with the application follows.

SEQUENCE LISTING (10 sequences)

SEQ ID NO: 1 - DNA, 20 bp, Artificial Sequence
  Synthetic Polynucleotide
ttcagccaaacgaccatctg

SEQ ID NO: 2 - DNA, 21 bp, Artificial Sequence
  Synthetic Polynucleotide
gaaccacactcggaccacatc

SEQ ID NO: 3 - DNA, 20 bp, Artificial Sequence
  Synthetic Polynucleotide
caccagtcccaaaggcaaac

SEQ ID NO: 4 - DNA, 20 bp, Artificial Sequence
  Synthetic Polynucleotide
gccttctgcgtcacaccatt

SEQ ID NO: 5 - DNA, 23 bp, Artificial Sequence
  Synthetic Polynucleotide
cacagaggagggaactgaatgac

SEQ ID NO: 6 - DNA, 20 bp, Artificial Sequence
  Synthetic Polynucleotide
aactcttcggctgcctctga

SEQ ID NO: 7 - DNA, 24 bp, Artificial Sequence
  Synthetic Polynucleotide
tggacactcacatgggagtcaaga

SEQ ID NO: 8 - DNA, 20 bp, Artificial Sequence
  Synthetic Polynucleotide
cgactgttgactgcaatgca

SEQ ID NO: 9 - DNA, 20 bp, Artificial Sequence
  Synthetic Polynucleotide
ctggaacggtgaaggtgaca

SEQ ID NO: 10 - DNA, 20 bp, Artificial Sequence
  Synthetic Polynucleotide
cggccacattgtgaactttg